European Patent Application EP 4 296 356 A1, published December 27, 2023. Title: MICRORNAS FROM FORSYTHIAE FRUCTUS-ASTRAGALI RADIX COMPOUND TRADITIONAL CHINESE MEDICINE DECOCTION AS WELL AS PREPARATION METHOD AND USE THEREOF. Applicant: NANTONG UNIVERSITY. The sequence listing filed with the application follows.

SEQUENCE LISTING (15 sequences)

SEQ ID NO: 1 - RNA, 28 nt, Artificial Sequence
ccagcacuaaugcaccggaucccaucag

SEQ ID NO: 2 - RNA, 25 nt, Artificial Sequence
ugggaaguccucguguuguaccccu

SEQ ID NO: 3 - RNA, 28 nt, Artificial Sequence
gccuucgaugucggcucuuccuaucauu

SEQ ID NO: 4 - RNA, 29 nt, Artificial Sequence
ucguccagcgguuaggauaucuggcuuuc

SEQ ID NO: 5 - RNA, 24 nt, Artificial Sequence
gcggaucuuggugguaguagcaaa

SEQ ID NO: 6 - RNA, 30 nt, Artificial Sequence
cucgggaaaaggauuggcucugagggcugg

SEQ ID NO: 7 - RNA, 25 nt, Artificial Sequence
acacaugcaagucgaacguuguuuu

SEQ ID NO: 8 - RNA, 28 nt, Artificial Sequence
gugugcaccggucgucucgucccuucug

SEQ ID NO: 9 - RNA, 24 nt, Artificial Sequence
ucugggugguguaguugguuauca

SEQ ID NO: 10 - RNA, 20 nt, Artificial Sequence
cguuucacgucggguucacc

SEQ ID NO: 11 - RNA, 23 nt, Artificial Sequence
gugguuaggacaucgucuuuuca

SEQ ID NO: 12 - RNA, 26 nt, Artificial Sequence
gucuguaguucgauccugcauggggg

SEQ ID NO: 13 - RNA, 20 nt, Artificial Sequence
uggcgcuagaaggagggccu

SEQ ID NO: 14 - RNA, 21 nt, Artificial Sequence
uuuggauugaagggagcucua

SEQ ID NO: 15 - RNA, 20 nt, Artificial Sequence
cuuggauugaagggagcucu